European Patent Specification EP 3 555 271 B1, published October 11, 2023. Title: ARYLALKYLAMINE N-ACETYLTRANSFERASE AND USES THEREOF. Applicant: Danmarks Tekniske Universitet. The sequence listing filed with the application follows.

SEQUENCE LISTING (6 sequences)

SEQ ID NO: 1 - protein, 182 aa, Streptomyces griseofuscus
MNTFRTATARDIPDVAATLTEAFATDPPTQWVFPDGTAAVSRFFTHVADRVHTAGGIVELLPDRAAMIALPPHVRLPGEAADGRQAEIQRRLADRHPLTPHYYLLFYGVRTAHQGSGLGGRMLARLTSRADRDRVGTYTEASTWRGARLMLRHGFHATRPLRLPDGPSMFPLWRDPIHDHSD

SEQ ID NO: 2 - protein, 207 aa, Bos taurus
MSTPSIHCLKPSPLHLPSGIPGSPGRQRRHTLPANEFRCLTPEDAAGVFEIEREAFISVSGNCPLNLDEVRHFLTLCPELSLGWFVEGRLVAFIIGSLWDEERLTQESLTLHRPGGRTAHLHALAVHHSFRQQGKGSVLLWRYLQHAGGQPAVRRAVLMCEDALVPFYQRFGFHPAGPCAVVVGSLTFTEMHCSLRGHAALRRNSDR

SEQ ID NO: 3 - protein, 205 aa, Gallus gallus
MPVLGAVPFLKPTPLQGPRNSPGRQRRHTLPASEFRCLSPEDAVSVFEIEREAFISVSGDCPLHLDEIRHFLTLCPELSLGWFEEGRLVAFIIGSLWDQDRLSQAALTLHNPRGTAVHIHVLAVHRTFRQQGKGSILMWRYLQYLRCLPCARRAVLMCEDFLVPFYEKCGFVAVGPCQVTVGTLAFTEMQHEVRGHAFMRRNSGC

SEQ ID NO: 4 - protein, 207 aa, Oryctolagus cuniculus
MSTLSTQPLKPKALHPPPGSPESPGHQRRHTLPASEFRCLTPEDAAGVFEIEREAFMSVSGSCPLYLDEIRHFLTLCPELSLGWFQEGRLVAFIIGSLWDKERLTQESLTLHRPGGRVAHLHVLAVHRACRQQGKGSVLLWRYLQHLGGQRAVRRAVLMCEDALVPFYERLGFRAVGPCAVTVGSLAFTELQCSVRGHACLRRKSGC

SEQ ID NO: 5 - protein, 205 aa, Mus musculus
MLNINSLKPEALHLPLGTSEFLGCQRRHTLPASEFRCLTPEDATSAFEIEREAFISVSGTCPLYLDEIRHFLTLCPELSLGWFEEGCLVAFIIGSLWDKERLTQESLTLHRPGGRTAHLHVLAVHRTFRQQGKGSVLLWRYLHHLGSQPAVRRAVLMCEDALVPFYEKFGFQAVGPCAITVGSLTFTELQCSLRCHAFLRRNSGC

SEQ ID NO: 6 - protein, 207 aa, Homo sapiens
MSTQSTHPLKPEAPRLPPGIPESPSCQRRHTLPASEFRCLTPEDAVSAFEIEREAFISVLGVCPLYLDEIRHFLTLCPELSLGWFEEGCLVAFIIGSLWDKERLMQESLTLHRSGGHIAHLHVLAVHRAFRQQGRGPILLWRYLHHLGSQPAVRRAALMCEDALVPFYERFSFHAVGPCAITVGSLTFMELHCSLRGHPFLRRNSGC